European Patent Application EP 4 803 541 A1, published September 9, 2026. Title: 抗GH单域抗体及其应用. Applicant: 长春金赛药业有限责任公司. Application CN. The sequence listing filed with the application follows.

SEQUENCE LISTING (53 sequences)

SEQ ID NO: 1 - protein, 142 aa, synthetic construct
  source 1..142: note = WT (with tag)
MQVQLVESGGGLAQAGGSLRLSCAVSGMPEFARAMGWFRQAPGKERELLAAIEGIGATTYYADSVKGRFTISRDDAANTVLLQMNSLKPDDTAVYYCAAAFSVTIPTRARHWVDWGPGTLVTVSSDDDDKSGGGGSHHHHHH

SEQ ID NO: 2 - protein, 142 aa, synthetic construct
  source 1..142: note = M8
MQVQLVESGGGLAQAGGSLRLSCAVSGMPEFARAMGWFRQAPGKERELLAAIEGIGATTYYADSVKGRFTISRDDAANTVLLQMNSLKPDDTAVYYCAAAFSVTIPTRARHWVYWGPGTLVTVSSDDDDKSGGGGSHHHHHH

SEQ ID NO: 3 - protein, 142 aa, synthetic construct
  source 1..142: note = M11
MQVQLVESGGGLAQAGGSLRLSCAVSGMPEFARAMGWFRQAPGKERELLAAIEGIGATTYYADSVKGRFTISRDDAANTVLLQMNSLKPDDTAVYYCAAAFSVTIPTRARHWVDWGQGTLVTVSSDDDDKSGGGGSHHHHHH

SEQ ID NO: 4 - protein, 142 aa, synthetic construct
  source 1..142: note = M20
MQVQLVESGGGLAQAGGSLRLSCAVSGMPEFARAMGWFRQAPGKERELVAAIEGIGATTYYADSVKGRFTISRDDAANTVLLQMNSLKPDDTAVYYCAAAFSVTIPTRARHWVDWGPGTLVTVSSDDDDKSGGGGSHHHHHH

SEQ ID NO: 5 - protein, 142 aa, synthetic construct
  source 1..142: note = M22
MQVQLVESGGGKAQAGGSLRLSCAVSGMPEFARAMGWFRQAPGKERELLAAIEGIGATTYYADSVKGRFTISRDDAANTVLLQMNSLKPDDTAVYYCAAAFSVTIPTRARHWVDWGPGTLVTVSSDDDDKSGGGGSHHHHHH

SEQ ID NO: 6 - protein, 142 aa, synthetic construct
  source 1..142: note = M24
MQVQLVESGGGLAQAGGSLRLSCAVSGMPEFARAMGWFRQAPGKERELLAAIEGIGATTYYADSVKGRFTISRDDAANTVLLQMNSLKPDDTAVYYCAAAFSVTIPTRARHFVDWGPGTLVTVSSDDDDKSGGGGSHHHHHH

SEQ ID NO: 7 - protein, 142 aa, synthetic construct
  source 1..142: note = M25
MQVQLVESGGGLAQAGGSLRLSCAVSGMPEFARAMGWFRQAPGKERELLAAIEGIGATTYYADSVKGRFTISRDDAANTVLLQMNSLKPDDTAVYYCAAAFSVTIPTRARHWDDWGPGTLVTVSSDDDDKSGGGGSHHHHHH

SEQ ID NO: 8 - protein, 142 aa, synthetic construct
  source 1..142: note = M27
MQVQLVESGGGLAQAGGSLRLSCAVSGMTEFARAMGWFRQAPGKERELLAAIEGIGATTYYADSVKGRFTISRDDAANTVLLQMNSLKPDDTAVYYCAAAFSVTIPTRARHWVDWGPGTLVTVSSDDDDKSGGGGSHHHHHH

SEQ ID NO: 9 - protein, 142 aa, synthetic construct
  source 1..142: note = M28
MQVQLVESGGGLAQAGGSLTLSCAVSGMPEFARAMGWFRQAPGKERELLAAIEGIGATTYYADSVKGRFTISRDDAANTVLLQMNSLKPDDTAVYYCAAAFSVTIPTRARHWVDWGPGTLVTVSSDDDDKSGGGGSHHHHHH

SEQ ID NO: 10 - protein, 142 aa, synthetic construct
  source 1..142: note = M29
MQVQLVESGGGLAQAGGSLRLSCAVSGMPEFARAMGWFRQAPGKERELLAAIEGIGAKTYYADSVKGRFTISRDDAANTVLLQMNSLKPDDTAVYYCAAAFSVTIPTRARHWVDWGPGTLVTVSSDDDDKSGGGGSHHHHHH

SEQ ID NO: 11 - protein, 142 aa, synthetic construct
  source 1..142: note = M31
MQVQLVESGGGLAQAGGSLRLSCAVSGMPEFARAMGWFRQAPGKERELLAAIEGIGATTYYADSVKGRFTISRDDAANTVLLQMNSLKPDDTAVYYCAAAFSVTIPTRAEHWVDWGPGTLVTVSSDDDDKSGGGGSHHHHHH

SEQ ID NO: 12 - protein, 142 aa, synthetic construct
  source 1..142: note = M33
MQVQLVESGGGLAQAGGSLRLSCAVSGMPEFARAMGWFRQAPGKERELLAAIEGIGDTTYYADSVKGRFTISRDDAANTVLLQMNSLKPDDTAVYYCAAAFSVTIPTRARHWVDWGPGTLVTVSSDDDDKSGGGGSHHHHHH

SEQ ID NO: 13 - protein, 142 aa, synthetic construct
  source 1..142: note = M34
MQVQLVESGGGLAQAGGSLRLSCAVSGMPEFARAMGWFRQAPGKERELLAAIEGIGATTYYADSVKGRFTISRDDAASTVLLQMNSLKPDDTAVYYCAAAFSVTIPTRARHWVDWGPGTLVTVSSDDDDKSGGGGSHHHHHH

SEQ ID NO: 14 - protein, 142 aa, synthetic construct
  source 1..142: note = M45
MQVQLVESGGGLAQAGGSLRLSCAVSGMPEFARAMGWFRQAPGKERELLAAIEGIGATTYYADSVKGRFTISRDDAANTVLLQMNSLKPDDTAVYYCAAAFSVTIPTRARHWVDWGPGTLVTVSSDDDDKSGGRGSHHHHHH

SEQ ID NO: 15 - protein, 142 aa, synthetic construct
  source 1..142: note = M50
MQVQLVESGGGLAQPGGSLRLSCAVSGMPEFARAMGWFRQAPGKERELLAAIEGIGATTYYADSVKGRFTISRDDAANTVLLQMNSLKPDDTAVYYCAAAFSVTIPTRARHWVDWGPGTLVTVSSDDDDKSGGGGSHHHHHH

SEQ ID NO: 16 - protein, 142 aa, synthetic construct
  source 1..142: note = M53
MQVQLVESGGGLAQAGGSLRLSCAVSGMPEFARAMGWFRQAPGKERELLAAIEGIGDTTYYADSVKGRFTISRDDAANTVLLQMNSLKPDDTAVYYCAAAFSVTIPTRAEHWVDWGPGTLVTVSSDDDDKSGGGGSHHHHHH

SEQ ID NO: 17 - protein, 142 aa, synthetic construct
  source 1..142: note = M59
MQVQLVESGGGLAQAGGSLRLSCAVSGMTEFARAMGWFRQAPGKERELLAAIEGIGDTTYYADSVKGRFTISRDDAANTVLLQMNSLKPDDTAVYYCAAAFSVTIPTRARHWVDWGPGTLVTVSSDDDDKSGGGGSHHHHHH

SEQ ID NO: 18 - protein, 142 aa, synthetic construct
  source 1..142: note = M64
MQVQLVESGGGLAQPGGSLRLSCAVSGMPEFARAMGWFRQAPGKERELLAAIEGIGATTYYADSVKGRFTISRDDAANTVLLQMNSLKPDDTAVYYCAAAFSVTIPTRARHWVDWGPGTLVTVSSDDDDKSGGRGSHHHHHH

SEQ ID NO: 19 - protein, 142 aa, synthetic construct
  source 1..142: note = M66
MQVQLVESGGGLAQPGGSLRLSCAVSGMTEFARAMGWFRQAPGKERELLAAIEGIGATTYYADSVKGRFTISRDDAANTVLLQMNSLKPDDTAVYYCAAAFSVTIPTRARHWVDWGPGTLVTVSSDDDDKSGGGGSHHHHHH

SEQ ID NO: 20 - protein, 142 aa, synthetic construct
  source 1..142: note = M67
MQVQLVESGGGLAQPGGSLRLSCAVSGMPEFARAMGWFRQAPGKERELLAAIEGIGATTYYADSVKGRFTISRDDAANTVLLQMNSLKPDDTAVYYCAAAFSVTIPTRARHWVDWGQGTLVTVSSDDDDKSGGGGSHHHHHH

SEQ ID NO: 21 - protein, 142 aa, synthetic construct
  source 1..142: note = M68
MQVQLVESGGGLAQPGGSLTLSCAVSGMPEFARAMGWFRQAPGKERELLAAIEGIGATTYYADSVKGRFTISRDDAANTVLLQMNSLKPDDTAVYYCAAAFSVTIPTRARHWVDWGPGTLVTVSSDDDDKSGGGGSHHHHHH

SEQ ID NO: 22 - protein, 142 aa, synthetic construct
  source 1..142: note = M69
MQVQLVESGGGLAQAGGSLRLSCAVSGMTEFARAMGWFRQAPGKERELLAAIEGIGATTYYADSVKGRFTISRDDAANTVLLQMNSLKPDDTAVYYCAAAFSVTIPTRARHWVDWGPGTLVTVSSDDDDKSGGRGSHHHHHH

SEQ ID NO: 23 - protein, 142 aa, synthetic construct
  source 1..142: note = M70
MQVQLVESGGGLAQPGGSLRLSCAVSGMPEFARAMGWFRQAPGKERELLAAIEGIGATTYYADSVKGRFTISRDDAANTVLLQMNSLKPDDTAVYYCAAAFSVTIPTRAEHWVDWGPGTLVTVSSDDDDKSGGGGSHHHHHH

SEQ ID NO: 24 - protein, 142 aa, synthetic construct
  source 1..142: note = M71
MQVQLVESGGGLAQAGGSLRLSCAVSGMPEFARAMGWFRQAPGKERELLAAIEGIGDTTYYADSVKGRFTISRDDAANTVLLQMNSLKPDDTAVYYCAAAFSVTIPTRAEHWVDWGQGTLVTVSSDDDDKSGGGGSHHHHHH

SEQ ID NO: 25 - protein, 142 aa, synthetic construct
  source 1..142: note = M72
MQVQLVESGGGLAQAGGSLRLSCAVSGMPEFARAMGWFRQAPGKERELLAAIEGIGDTTYYADSVKGRFTISRDDAANTVLLQMNSLKPDDTAVYYCAAAFSVTIPTRARHFVYWGPGTLVTVSSDDDDKSGGGGSHHHHHH

SEQ ID NO: 26 - protein, 142 aa, synthetic construct
  source 1..142: note = M74
MQVQLVESGGGLAQAGGSLRLSCAVSGMPEFARAMGWFRQAPGKERELLAAIEGIGDTTYYADSVKGRFTISRDDAANTVLLQMNSLKPDDTAVYYCAAAFSVTIPTRAEHWVDWGPGTLVTVSSDDDDKSGGRGSHHHHHH

SEQ ID NO: 27 - protein, 142 aa, synthetic construct
  source 1..142: note = M75
MQVQLVESGGGLAQAGGSLRLSCAVSGMPEFARAMGWFRQAPGKERELLAAIEGIGDTTYYADSVKGRFTISRDDAANTVLLQMNSLKPDDTAVYYCAAAFSVTIPTRAEHWVYWGPGTLVTVSSDDDDKSGGGGSHHHHHH

SEQ ID NO: 28 - protein, 142 aa, synthetic construct
  source 1..142: note = M76
MQVQLVESGGGLAQAGGSLRLSCAVSGMPEFARAMGWFRQAPGKERELLAAIEGIGDTTYYADSVKGRFTISRDDAANTVLLQMNSLKPDDTAVYYCAAAFSVTIPTRARHFVDWGPGTLVTVSSDDDDKSGGRGSHHHHHH

SEQ ID NO: 29 - protein, 142 aa, synthetic construct
  source 1..142: note = M77
MQVQLVESGGGLAQAGGSLRLSCAVSGMPEFARAMGWFRQAPGKERELLAAIEGIGDTTYYADSVKGRFTISRDDAANTVLLQMNSLKPDDTAVYYCAAAFSVTIPTRAEHFVDWGPGTLVTVSSDDDDKSGGGGSHHHHHH

SEQ ID NO: 30 - protein, 142 aa, synthetic construct
  source 1..142: note = M78
MQVQLVESGGGLAQAGGSLRLSCAVSGMPEFARAMGWFRQAPGKERELLAAIEGIGDTTYYADSVKGRFTISRDDAANTVLLQMNSLKPDDTAVYYCAAAFSVTIPTRARHWVYWGPGTLVTVSSDDDDKSGGRGSHHHHHH

SEQ ID NO: 31 - protein, 142 aa, synthetic construct
  source 1..142: note = M79
MQVQLVESGGGLAQAGGSLRLSCAVSGMPEFARAMGWFRQAPGKERELVAAIEGIGDTTYYADSVKGRFTISRDDAANTVLLQMNSLKPDDTAVYYCAAAFSVTIPTRAEHWVDWGPGTLVTVSSDDDDKSGGGGSHHHHHH

SEQ ID NO: 32 - protein, 142 aa, synthetic construct
  source 1..142: note = M81
MQVQLVESGGGLAQAGGSLRLSCAVSGMPEFARAMGWFRQAPGKERELLAAIEGIGDTTYYADSVKGRFTISRDDAANTVLLQMNSLKPDDTAVYYCAAAFSVTIPTRAEHWVDWGQGTLVTVSSDDDDKSGGRGSHHHHHH

SEQ ID NO: 33 - protein, 142 aa, synthetic construct
  source 1..142: note = M82
MQVQLVESGGGLAQAGGSLRLSCAVSGMPEFARAMGWFRQAPGKERELLAAIEGIGDTTYYADSVKGRFTISRDDAANTVLLQMNSLKPDDTAVYYCAAAFSVTIPTRAEHWVYWGPGTLVTVSSDDDDKSGGRGSHHHHHH

SEQ ID NO: 34 - protein, 142 aa, synthetic construct
  source 1..142: note = M83
MQVQLVESGGGLAQAGGSLRLSCAVSGMPEFARAMGWFRQAPGKERELLAAIEGIGDTTYYADSVKGRFTISRDDAANTVLLQMNSLKPDDTAVYYCAAAFSVTIPTRAEHFVDWGQGTLVTVSSDDDDKSGGGGSHHHHHH

SEQ ID NO: 35 - protein, 142 aa, synthetic construct
  source 1..142: note = M88
MQVQLVESGGGLAQAGGSLRLSCAVSGMPEFARAMGWFRQAPGKERELVAAIEGIGDTTYYADSVKGRFTISRDDAANTVLLQMNSLKPDDTAVYYCAAAFSVTIPTRAEHWVDWGPGTLVTVSSDDDDKSGGRGSHHHHHH

SEQ ID NO: 36 - protein, 142 aa, synthetic construct
  source 1..142: note = M89
MQVQLVESGGGLAQAGGSLRLSCAVSGMPEFARAMGWFRQAPGKERELLAAIEGIGDTTYYADSVKGRFTISRDDAANTVLLQMNSLKPDDTAVYYCAAAFSVTIPTRAEHFVDWGPGTLVTVSSDDDDKSGGRGSHHHHHH

SEQ ID NO: 37 - protein, 125 aa, synthetic construct
  source 1..125: note = WT
MQVQLVESGGGLAQAGGSLRLSCAVSGMPEFARAMGWFRQAPGKERELLAAIEGIGATTYYADSVKGRFTISRDDAANTVLLQMNSLKPDDTAVYYCAAAFSVTIPTRARHWVDWGPGTLVTVSS

SEQ ID NO: 38 - protein, 5 aa, synthetic construct
  source 1..5: note = recognition sequence of Enterokinase
DDDDK

SEQ ID NO: 39 - protein, 6 aa, synthetic construct
  source 1..6: note = His tag
HHHHHH

SEQ ID NO: 40 - protein, 6 aa, synthetic construct
  source 1..6: note = Linker-1
SGGGGS

SEQ ID NO: 41 - protein, 6 aa, unidentified
  source 1..6: note = Linker-2
SGGRGS

SEQ ID NO: 42 - protein, 5 aa, synthetic construct
  source 1..5: note = CDR1
ARAMG

SEQ ID NO: 43 - protein, 17 aa, synthetic construct
  source 1..17: note = CDR2
AIEGIGATTYYADSVKG

SEQ ID NO: 44 - protein, 17 aa, synthetic construct
  source 1..17: note = CDR2
AIEGIGAKTYYADSVKG

SEQ ID NO: 45 - protein, 17 aa, synthetic construct
  source 1..17: note = CDR2
AIEGIGDTTYYADSVKG

SEQ ID NO: 46 - protein, 15 aa, synthetic construct
  source 1..15: note = CDR3
AFSVTIPTRARHWVD

SEQ ID NO: 47 - protein, 15 aa, synthetic construct
  source 1..15: note = CDR3
AFSVTIPTRARHWVY

SEQ ID NO: 48 - protein, 15 aa, synthetic construct
  source 1..15: note = CDR3
AFSVTIPTRARHFVD

SEQ ID NO: 49 - protein, 15 aa, synthetic construct
  source 1..15: note = CDR3
AFSVTIPTRARHWDD

SEQ ID NO: 50 - protein, 15 aa, synthetic construct
  source 1..15: note = CDR3
AFSVTIPTRAEHWVD

SEQ ID NO: 51 - protein, 15 aa, synthetic construct
  source 1..15: note = CDR3
AFSVTIPTRARHFVY

SEQ ID NO: 52 - protein, 15 aa, synthetic construct
  source 1..15: note = CDR3
AFSVTIPTRAEHWVY

SEQ ID NO: 53 - protein, 15 aa, synthetic construct
  source 1..15: note = CDR3
AFSVTIPTRAEHFVD